European Patent Specification EP 3 404 042 B1, published June 11, 2025. Title: A MONOCLONAL ANTIBODY FnAb8 AND USE THEREOF. Applicant: SHANGHAI JIAO TONG UNIVERSITY. The sequence listing filed with the application follows.

SEQUENCE LISTING (36 sequences)

SEQ ID NO: 1 - protein, 365 aa, Homo sapiens
MGVPRPQPWALGLLLFLLPGSLGAESHLSLLYHLTAVSSPAPGTPAFWVSGWLGPQQYLSYNSLRGEAEPCGAWVWENQVSWYWEKETTDLRIKEKLFLEAFKALGGKGPYTLQGLLGCELGPDNTSVPTAKFALNGEEFMNFDLKQGTWGGDWPEALAISQRWQQQDKAANKELTFLLFSCPHRLREHLERGRGNLEWKEPPSMRLKARPSSPGFSVLTCSAFSFYPPELQLRFLRNGLAAGTGQGDFGPNSDGSFHASSSLTVKSGDEHHYCCIVQHAGLAQPLRVELESPAKSSVLVVGIVIGVLLLTAAAVGGALLWRRMRSGLPAPWISLRGDDTGVLLPTPGEAQDADLKDVNVIPATA

SEQ ID NO: 2 - protein, 30 aa, Artificial sequence
  Polypeptide
HGEGTFTSDVSSYLEEQAAKEFIAWLVKGG

SEQ ID NO: 3 - DNA, 24 bp, Artificial sequence
  Polynucleotide
ggatacaccttcaccggctactat

SEQ ID NO: 4 - protein, 8 aa, Artificial sequence
  Polypeptide
GYTFTGYY

SEQ ID NO: 5 - DNA, 24 bp, Artificial sequence
  Polynucleotide
atcagccctcacagtggtggcaca

SEQ ID NO: 6 - protein, 8 aa, Artificial sequence
  Polypeptide
ISPHSGGT

SEQ ID NO: 7 - DNA, 27 bp, Artificial sequence
  Polynucleotide
gcgcgcggtgtttacggtatggatcgt

SEQ ID NO: 8 - protein, 9 aa, Artificial sequence
  Polypeptide
ARGVYGMDR

SEQ ID NO: 9 - DNA, 348 bp, Artificial sequence
  Polynucleotide
caggtgcagctggtgcagtctggggctgaggtgaagaagcctggggcctcagtgaaggtctcctgcaagacttctggatacaccttcaccggctactatatacactgggtgcgacaggcccctggacaagggcttgagtggatgggacatatcagccctcacagtggtggcacagactatgcacagaagtttcagggcagggtcaccatgaccagggacacgtccatcagcacagcctacatggagctgagcaggctgagatctgacgacactgccgtgtattactgtgcgcgcggtgtttacggtatggatcgttggggtcaaggtactctggtgaccgtctcctca

SEQ ID NO: 10 - protein, 116 aa, Artificial sequence
  Polypeptide
QVQLVQSGAEVKKPGASVKVSCKTSGYTFTGYYIHWVRQAPGQGLEWMGHISPHSGGTDYAQKFQGRVTMTRDTSISTAYMELSRLRSDDTAVYYCARGVYGMDRWGQGTLVTVSS

SEQ ID NO: 11 - protein, 295 aa, Artificial sequence
  Polypeptide
HGEGTFTSDVSSYLEEQAAKEFIAWLVKGGGGGGGSGGGGSGGGGSQAVLTQPPSASGTPGQRVTISCSGSSSNIGSNSVNWYQQLPGTAPKLLIYSNNQRPSGVPDRFSGSKSGTSASLAISGLQSEDEADYYCAAWDDSLNGRVLFGGGTKLTVLGSRGGGGSGGGGSGGGGSLEMAQVQLVQSGAEVKKPGASVKVSCKTSGYTFTGYYIHWVRQAPGQGLEWMGHISPHSGGTDYAQKFQGRVTMTRDTSISTAYMELSRLRSDDTAVYYCARGVYGMDRWGQGTLVTVSS

SEQ ID NO: 12 - protein, 291 aa, Artificial sequence
  Polypeptide
HGEGTFTSDVSSYLEEQAAKEFIAWLVKGGGGGGGSGGGGSGGGGSDIQLTQSPSSLSASVGDRVTLTCQATQDIDNNLNWYQQKPGKAPKLLIYDASNLETGVPSRFSGSGSGTDFTFTISDLQPEDVATYYCQQYYNLPLTFGGGTKVDIKRSRGGGGSGGGGSGGGGSLEMAEVQLVQSGAEVKKPGASVKVSCKASGYTFTSYDINWVRQATGQGLEWMGWMNPNSGNTGYAQKFQGRVTMTRNTSISTAYMELSSLRSEDTAVYYCARGVDLGDGWGQGTLVTVSS

SEQ ID NO: 13 - DNA, 24 bp, Artificial sequence
  Polynucleotide
agctccaacatcggaagtaatagt

SEQ ID NO: 14 - protein, 8 aa, Artificial sequence
  Polypeptide
SSNIGSNS

SEQ ID NO: 15 - DNA, 9 bp, Artificial sequence
  Polynucleotide
agtaataat

SEQ ID NO: 16 - protein, 3 aa, Artificial sequence
  Polypeptide
SNN

SEQ ID NO: 17 - DNA, 36 bp, Artificial sequence
  Polynucleotide
gcagcgtgggatgacagcctgaatggccgtgtacta

SEQ ID NO: 18 - protein, 12 aa, Artificial sequence
  Polypeptide
AAWDDSLNGRVL

SEQ ID NO: 19 - DNA, 333 bp, Artificial sequence
  Polynucleotide
caggctgtgctgactcagccaccctcagcgtctgggacccccgggcagagggtcaccatctcttgttctggaagcagctccaacatcggaagtaatagtgtaaactggtaccagcagctcccaggaacggcccccaaactcctcatctatagtaataatcagcggccctcaggggtccctgaccgattctctggctccaagtctggcacctcagcctccctggccatcagtgggctccagtctgaggatgaggctgattattactgtgcagcgtgggatgacagcctgaatggccgtgtactattcggcggagggaccaagctgaccgtccta

SEQ ID NO: 20 - protein, 111 aa, Artificial sequence
  Polypeptide
QAVLTQPPSASGTPGQRVTISCSGSSSNIGSNSVNWYQQLPGTAPKLLIYSNNQRPSGVPDRFSGSKSGTSASLAISGLQSEDEADYYCAAWDDSLNGRVLFGGGTKLTVL

SEQ ID NO: 21 - DNA, 24 bp, Artificial sequence
  Polynucleotide
ggatacaccttcaccagttatgat

SEQ ID NO: 22 - protein, 8 aa, Artificial sequence
  Polypeptide
GYTFTSYD

SEQ ID NO: 23 - DNA, 24 bp, Artificial sequence
  Polynucleotide
atgaaccctaacagtggtaacaca

SEQ ID NO: 24 - protein, 8 aa, Artificial sequence
  Polypeptide
MNPNSGNT

SEQ ID NO: 25 - DNA, 27 bp, Artificial sequence
  Polynucleotide
gcgcgcggtgttgacctgggtgatggt

SEQ ID NO: 26 - protein, 9 aa, Artificial sequence
  Polypeptide
ARGVDLGDG

SEQ ID NO: 27 - DNA, 348 bp, Artificial sequence
  Polynucleotide
gaggtccagctggtgcagtctggggctgaggtgaagaagcctggggcctcagtgaaggtctcctgcaaggcttctggatacaccttcaccagttatgatatcaactgggtgcgacaggccactggacaagggcttgagtggatgggatggatgaaccctaacagtggtaacacaggctatgcacagaagttccagggcagagtcaccatgaccaggaacacctccataagcacagcctacatggagctgagcagcctgagatctgaggacacggccgtgtattactgtgcgcgcggtgttgacctgggtgatggttggggtcaaggtactctggtgaccgtctcctca

SEQ ID NO: 28 - protein, 116 aa, Artificial sequence
  Polypeptide
EVQLVQSGAEVKKPGASVKVSCKASGYTFTSYDINWVRQATGQGLEWMGWMNPNSGNTGYAQKFQGRVTMTRNTSISTAYMELSSLRSEDTAVYYCARGVDLGDGWGQGTLVTVSS

SEQ ID NO: 29 - DNA, 18 bp, Artificial sequence
  Polynucleotide
caggacattgacaacaac

SEQ ID NO: 30 - protein, 6 aa, Artificial sequence
  Polypeptide
QDIDNN

SEQ ID NO: 31 - DNA, 9 bp, Artificial sequence
  Polynucleotide
gatgcgtcc

SEQ ID NO: 32 - protein, 3 aa, Artificial sequence
  Polypeptide
DAS

SEQ ID NO: 33 - DNA, 27 bp, Artificial sequence
  Polynucleotide
caacagtattacaatctgcctctgact

SEQ ID NO: 34 - protein, 9 aa, Artificial sequence
  Polypeptide
QQYYNLPLT

SEQ ID NO: 35 - DNA, 321 bp, Artificial sequence
  Polynucleotide
gacatccagttgacccagtctccatcctccctgtctgcatccgttggcgacagagtcaccctcacttgccaggcgactcaggacattgacaacaacttaaattggtatcaacaaaagccggggaaagcccctaagctcctgatctacgatgcgtccaatttggaaacaggagtcccgtcacggttcagcgggagtggatctgggacagattttactttcaccattagtgacctacagcctgaagatgttgcaacatattactgtcaacagtattacaatctgcctctgactttcggcggagggaccaaagtggatatcaaa

SEQ ID NO: 36 - protein, 107 aa, Artificial sequence
  Polypeptide
DIQLTQSPSSLSASVGDRVTLTCQATQDIDNNLNWYQQKPGKAPKLLIYDASNLETGVPSRFSGSGSGTDFTFTISDLQPEDVATYYCQQYYNLPLTFGGGTKVDIK